European Patent Specification EP 3 322 437 B1, published January 17, 2024. Title: Novel glucagon derivative and a composition comprising a long acting conjugate of the same. Applicant: HANMI PHARM. CO., LTD. The sequence listing filed with the application follows.

SEQUENCE LISTING (48 sequences)

SEQ ID NO: 1 - protein, 29 aa, homo sapiens
HSQGTFTSDYSKYLDSRRAQDFVQWLMNT

SEQ ID NO: 2 - protein, 29 aa, Artificial Sequence
  glucagon derivative
HSQGTFTSDYSKYLDCDRAQDFVQWLMNT

SEQ ID NO: 3 - protein, 29 aa, Artificial Sequence
  glucagon derivative
HSQGTFTSDYSKYLDCERAQDFVQWLMNT

SEQ ID NO: 4 - protein, 29 aa, Artificial Sequence
  glucagon derivative
HSQGTFTSDYSKYLDSCDAQDFVQWLMNT

SEQ ID NO: 5 - protein, 29 aa, Artificial Sequence
  glucagon derivative
HSQGTFTSDYSKYLDSCEAQDFVQWLMNT

SEQ ID NO: 6 - protein, 29 aa, Artificial Sequence
  glucagon derivative
HSQGTFTSDYSKYLDSCEADDFVQWLMNT

SEQ ID NO: 7 - protein, 29 aa, Artificial Sequence
  glucagon derivative
YSQGTFTSDYSKYLDSCEADDFVQWLMNT

SEQ ID NO: 8 - protein, 29 aa, Artificial Sequence
  glucagon derivative
  MISC_FEATURE (2): Xaa is aminoisobutyric acid (Aib)
YXQGTFTSDYSKYLDSCDAQDFVQWLINT

SEQ ID NO: 9 - protein, 29 aa, Artificial Sequence
  glucagon derivative
  MISC_FEATURE (2): Xaa is aminoisobutyric acid (Aib)
YXQGTFTSDYSKYLDSCDAQDFVVWLINT

SEQ ID NO: 10 - protein, 29 aa, Artificial Sequence
  glucagon derivative
  MISC_FEATURE (2): Xaa is aminoisobutyric acid (Aib)
YXQGTFTSDYSKYLDSCDADDFVVWLINT

SEQ ID NO: 11 - protein, 29 aa, Artificial Sequence
  glucagon derivative
  MISC_FEATURE (2): Xaa is aminoisobutyric acid (Aib)
YXQGTFTSDYSKYLDEKCAKEFVQWLMNT

SEQ ID NO: 12 - protein, 30 aa, Artificial Sequence
  glucagon derivative
  MISC_FEATURE (2): Xaa is aminoisobutyric acid (Aib)
  MISC_FEATURE (16)..(20): amino acids at positions 16 and 20 form a ring
YXQGTFTSDYSKYLDEKRAKEFVQWLMNTC

SEQ ID NO: 13 - protein, 29 aa, Artificial Sequence
  glucagon derivative
  MISC_FEATURE (2): Xaa is aminoisobutyric acid (Aib)
YXQGTFTSDYSCYLDSRRAQDFVQWLMNT

SEQ ID NO: 14 - protein, 29 aa, Artificial Sequence
  glucagon derivative
  MISC_FEATURE (2): Xaa is aminoisobutyric acid (Aib)
YXQGTFTSDYSKYLDCKRAKEFVQWLMNT

SEQ ID NO: 15 - protein, 29 aa, Artificial Sequence
  glucagon derivative
  MISC_FEATURE (2): Xaa is aminoisobutyric acid (Aib)
YXQGTFTSDYSKYLCEKRAQDFVVWLMNT

SEQ ID NO: 16 - protein, 29 aa, Artificial Sequence
  glucagon derivative
  MISC_FEATURE (2): Xaa is aminoisobutyric acid (Aib)
YXQGTFTSDYSKYLDCRRAQVFVQWLMRT

SEQ ID NO: 17 - protein, 29 aa, Artificial Sequence
  glucagon derivative
  MISC_FEATURE (2): Xaa is aminoisobutyric acid (Aib)
YXQGTFTSDYSKYLDCVRAQDFVQWLMRT

SEQ ID NO: 18 - protein, 29 aa, Artificial Sequence
  glucagon derivative
  MISC_FEATURE (2): Xaa is aminoisobutyric acid (Aib)
YXQGTFTSDYSKYLDSRRACDFRLWLMNT

SEQ ID NO: 19 - protein, 29 aa, Artificial Sequence
  glucagon derivative
  MISC_FEATURE (2): Xaa is aminoisobutyric acid (Aib)
  MISC_FEATURE (16)..(20): amino acids at positions 16 and 20 form a ring
YXQGTFTSDYSKYLCEKRAKEFVQWLMNT

SEQ ID NO: 20 - protein, 29 aa, Artificial Sequence
  glucagon derivative
  MISC_FEATURE (2): Xaa is aminoisobutyric acid (Aib)
  MISC_FEATURE (16)..(20): amino acids at positions 16 and 20 form a ring
YXQGTFTSDYSKYLDECRAKEFVQWLMNT

SEQ ID NO: 21 - protein, 29 aa, Artificial Sequence
  glucagon derivative
  MISC_FEATURE (2): Xaa is aminoisobutyric acid (Aib)
  MISC_FEATURE (16)..(20): amino acids at positions 16 and 20 form a ring
YXQGTFTSDYSKYLDEKCAKEFVQWLMNT

SEQ ID NO: 22 - protein, 29 aa, Artificial Sequence
  glucagon derivative
  MISC_FEATURE (2): Xaa is aminoisobutyric acid (Aib)
  MISC_FEATURE (16)..(20): amino acids at positions 16 and 20 form a ring
YXQGTFTSDYSKYLDEKRCKEFVQWLMNT

SEQ ID NO: 23 - protein, 29 aa, Artificial Sequence
  glucagon derivative
  MISC_FEATURE (2): Xaa is aminoisobutyric acid (Aib)
  MISC_FEATURE (16)..(20): amino acids at positions 16 and 20 form a ring
YXQGTFTSDYSKYCDEKRAKEFVQWLMNT

SEQ ID NO: 24 - protein, 29 aa, Artificial Sequence
  glucagon derivative
  MISC_FEATURE (2): Xaa is aminoisobutyric acid (Aib)
  MISC_FEATURE (16)..(20): amino acids at positions 16 and 20 form a ring
YXQGTFTSDYSKCLDEKRAKEFVQWLMNT

SEQ ID NO: 25 - protein, 29 aa, Artificial Sequence
  glucagon derivative
  MISC_FEATURE (2): Xaa is aminoisobutyric acid (Aib)
  MISC_FEATURE (16)..(20): amino acids at positions 16 and 20 form a ring
YXQGTFTSDYSKYLDEKRAKCFVQWLMNT

SEQ ID NO: 26 - protein, 29 aa, Artificial Sequence
  glucagon derivative
  MISC_FEATURE (2): Xaa is aminoisobutyric acid (Aib)
  MISC_FEATURE (16)..(20): amino acids at positions 16 and 20 form a ring
WXQGTFTSDYSKYLDECRAKDFVQWLMNT

SEQ ID NO: 27 - protein, 29 aa, Artificial Sequence
  glucagon derivative
  MISC_FEATURE (2): Xaa is aminoisobutyric acid (Aib)
  MISC_FEATURE (16)..(20): amino acids at positions 16 and 20 form a ring
YXQGTFVSDYSKYLDECRAKDFVQWLMNT

SEQ ID NO: 28 - protein, 29 aa, Artificial Sequence
  glucagon derivative
  MISC_FEATURE (2): Xaa is aminoisobutyric acid (Aib)
  MISC_FEATURE (16)..(20): amino acids at positions 16 and 20 form a ring
WXQGTFVSDYSKYLDECRAKDFVQWLMNT

SEQ ID NO: 29 - protein, 29 aa, Artificial Sequence
  glucagon derivative
  MISC_FEATURE (2): Xaa is aminoisobutyric acid (Aib)
  MISC_FEATURE (16)..(20): amino acids at positions 16 and 20 form a ring
YXQGTFTSDYSKCLDERRAKDFVQWLMNT

SEQ ID NO: 30 - protein, 29 aa, Artificial Sequence
  glucagon derivative
  MISC_FEATURE (2): Xaa is aminoisobutyric acid (Aib)
  MISC_FEATURE (16)..(20): amino acids at positions 16 and 20 form a ring
WXQGTFTSDYSKCLDERRAKDFVQWLMNT

SEQ ID NO: 31 - protein, 29 aa, Artificial Sequence
  glucagon derivative
  MISC_FEATURE (2): Xaa is aminoisobutyric acid (Aib)
  MISC_FEATURE (17)..(21): amino acids at positions 17 and 21 form a ring
YXQGTFTSDYSKYLDCKRAKEFVQWLMNT

SEQ ID NO: 32 - protein, 28 aa, Artificial Sequence
  glucagon derivative
  MISC_FEATURE (15)..(19): amino acids at positions 15 and 19 form a ring
SQGTFTSDYSKYLDECRAKEFVQWLMNT

SEQ ID NO: 33 - protein, 29 aa, Artificial Sequence
  glucagon derivative
  MISC_FEATURE (2): Xaa is aminoisobutyric acid (Aib)
YXQGTFTSDYSKYLDSRRAQDFVQWLMNT

SEQ ID NO: 34 - protein, 29 aa, Artificial Sequence
  glucagon derivative
  MISC_FEATURE (2): Xaa is aminoisobutyric acid (Aib)
  MISC_FEATURE (16)..(20): amino acids at positions 16 and 20 form a ring
WXQGTFTSDYSKYCDERRAKEFVQWLMNT

SEQ ID NO: 35 - protein, 29 aa, Artificial Sequence
  glucagon derivative
  MISC_FEATURE (2): Xaa is aminoisobutyric acid (Aib)
  MISC_FEATURE (16)..(20): amino acids at positions 16 and 20 form a ring
YXQGTFTSDYSKYCDERRAKEFVQWLMNT

SEQ ID NO: 36 - protein, 29 aa, Artificial Sequence
  glucagon derivative
  MISC_FEATURE (2): Xaa is aminoisobutyric acid (Aib)
  MISC_FEATURE (16)..(20): amino acids at positions 16 and 20 form a ring
YXQGTFTSDCSKYLDERRAKEFVQWLMNT

SEQ ID NO: 37 - protein, 30 aa, Artificial Sequence
  glucagon derivative
  MISC_FEATURE (2): Xaa is aminoisobutyric acid (Aib)
  MISC_FEATURE (16)..(20): amino acids at positions 16 and 20 form a ring
YXQGTFTSDYSKYLDERRAKEFVQWLMNTC

SEQ ID NO: 38 - protein, 29 aa, Artificial Sequence
  glucagon derivative
  MISC_FEATURE (2): Xaa is aminoisobutyric acid (Aib)
  MISC_FEATURE (16)..(20): amino acids at positions 16 and 20 form a ring
YXQGTFCSDYSKYLDERRAKEFVQWLMNT

SEQ ID NO: 39 - protein, 29 aa, Artificial Sequence
  glucagon derivative
  MISC_FEATURE (2): Xaa is aminoisobutyric acid (Aib)
  MISC_FEATURE (16)..(20): amino acids at positions 16 and 20 form a ring
YXQGTFVSDCSKYLDERRAKDFVQWLMNT

SEQ ID NO: 40 - protein, 30 aa, Artificial Sequence
  glucagon derivative
  MISC_FEATURE (2): Xaa is aminoisobutyric acid (Aib)
  MISC_FEATURE (16)..(20): amino acids at positions 16 and 20 form a ring
YXQGTFVSDYSKYLDERRAKDFVQWLMNTC

SEQ ID NO: 41 - protein, 29 aa, Artificial Sequence
  glucagon derivative
  MISC_FEATURE (2): Xaa is aminoisobutyric acid (Aib)
  MISC_FEATURE (16)..(20): amino acids at positions 16 and 20 form a ring
YXQGTFCSDYSKYLDERRAKDFVQWLMNT

SEQ ID NO: 42 - protein, 29 aa, Artificial Sequence
  glucagon derivative
  MISC_FEATURE (2): Xaa is aminoisobutyric acid (Aib)
YXQGTFCSDYSKYLDSRRAQDFVQWLMNT

SEQ ID NO: 43 - protein, 29 aa, Artificial Sequence
  glucagon derivative
  MISC_FEATURE (2): Xaa is aminoisobutyric acid (Aib)
YXQGTFTSDCSKYLDSRRAQDFVQWLMNT

SEQ ID NO: 44 - protein, 30 aa, Artificial Sequence
  glucagon derivative
  MISC_FEATURE (2): Xaa is aminoisobutyric acid (Aib)
YXQGTFTSDYSKYLDSRRAQDFVQWLMNTC

SEQ ID NO: 45 - protein, 30 aa, Artificial Sequence
  glucagon derivative
  MISC_FEATURE (1): Xaa is histidine, desamino-histidyl, N-dimethyl-histidyl, beta-hydroxy imidazopropionyl, 4-imidazoacetyl, beta-carboxy imidazopropionyl, tryptophan, or tyrosine, or is absent
  MISC_FEATURE (2): Xaa is alpha-methyl-glutamic acid, aminoisobutyric acid (Aib), D-alanine, glycine, Sar (N-methylglycine), serine, or D-serine
  MISC_FEATURE (7): Xaa is threonine, valine, or cysteine
  MISC_FEATURE (10): Xaa is tyrosine or cysteine
  MISC_FEATURE (12): Xaa is lysine or cysteine
  MISC_FEATURE (13): Xaa is tyrosine or cysteine
  MISC_FEATURE (14): Xaa is leucine or cysteine
  MISC_FEATURE (15): Xaa is aspartic acid, glutamic acid, or cysteine
  MISC_FEATURE (16): Xaa is glutamic acid, aspartic acid, serine, alpha-methyl-glutamic acid, or cysteine, or is absent;
  MISC_FEATURE (17): Xaa is aspartic acid, glutamine, glutamic acid, lysine, arginine, serine, cysteine, or valine, or is absent
  MISC_FEATURE (18): Xaa is alanine, aspartic acid, glutamic acid, arginine, valine, or cysteine, or is absent
  MISC_FEATURE (19): Xaa is alanine, arginine, serine, valine, or cysteine, or is absent
  MISC_FEATURE (20): Xaa is lysine, histidine, glutamine, aspartic acid, lysine, arginine, alpha-methyl-glutamic acid, or cysteine, or is absent
  MISC_FEATURE (21): Xaa is aspartic acid, glutamic acid, leucine, valine, or cysteine, or is absent
  MISC_FEATURE (23): Xaa is isoleucine, valine, or arginine, or is absent
  MISC_FEATURE (24): Xaa is valine, arginine, alanine, cysteine, glutamic acid, lysine, glutamine, alpha-methyl-glutamic acid, or leucine, or is absent;
  MISC_FEATURE (27): Xaa is isoleucine, valine, alanine, lysine, methionine, glutamine, or arginine, or is absent
  MISC_FEATURE (28): Xaa is glutamine, lysine, asparagine, or arginine, or is absent
  MISC_FEATURE (29): Xaa is lysine, alanine, glycine, or threonine, or is absent
  MISC_FEATURE (30): Xaa is cysteine, or is absent
XXQGTFXSDXSXXXXXXXXXXFXXWLXXXX

SEQ ID NO: 46 - protein, 30 aa, Artificial Sequence
  glucagon derivative
  MISC_FEATURE (2): Xaa is aminoisobutyric acid (Aib)
  MISC_FEATURE (7): Xaa is threonine, valine, or cysteine
  MISC_FEATURE (10): Xaa is tyrosine or cysteine
  MISC_FEATURE (12): Xaa is lysine or cysteine
  MISC_FEATURE (15): Xaa is aspartic acid or cysteine
  MISC_FEATURE (16): Xaa is glutamic acid or serine
  MISC_FEATURE (17): Xaa is lysine or arginine
  MISC_FEATURE (20): Xaa is glutamine or lysine
  MISC_FEATURE (21): Xaa is aspartic acid or glutamic acid
  MISC_FEATURE (24): Xaa is valine or glutamine
  MISC_FEATURE (30): Xaa is cysteine or is absent
YXQGTFXSDXSXYLXXXRAXXFVXWLMNTX

SEQ ID NO: 47 - DNA, 34 bp, Artificial Sequence
  forward primer
cagcgacaccgaccgtccccccgtacttaaggcc

SEQ ID NO: 48 - DNA, 32 bp, Artificial Sequence
  reverse primer
ctaaccgactctcggggaagactgagctcgcc